European Patent Application EP 4 644 371 A1, published November 5, 2025. Title: 4-AMINOPIPERIDINE COMPOUND, LIPID NANOPARTICLES THEREOF AND PHARMACEUTICAL COMPOSITION CONTAINING THE SAME. Applicant: Astellas Pharma Inc. The sequence listing filed with the application follows.

SEQUENCE LISTING (5 sequences)

SEQ ID NO: 1 - DNA, 1071 bp, Homo sapiens
  source 1..1071: mol_type = other DNA
  misc_feature 1..1071: note = Human NeuroD1 Gene (CDS)
atgaccaaatcgtacagcgagagtgggctgatgggcgagcctcagccccaaggtcctccaagctggacagacgagtgtctcagttctcaggacgaggagcacgaggcagacaagaaggaggacgacctcgaaaccatgaacgcagaggaggactcactgaggaacgggggagaggaggaggacgaagatgaggacctggaagaggaggaagaagaggaagaggaggatgacgatcaaaagcccaagagacgcggccccaaaaagaagaagatgactaaggctcgcctggagcgttttaaattgagacgcatgaaggctaacgcccgggagcggaaccgcatgcacggactgaacgcggcgctagacaacctgcgcaaggtggtgccttgctattctaagacgcagaagctgtccaaaatcgagactctgcgcttggccaagaactacatctgggctctgtcggagatcctgcgctcaggcaaaagcccagacctggtctccttcgttcagacgctttgcaagggcttatcccaacccaccaccaacctggttgcgggctgcctgcaactcaatcctcggacttttctgcctgagcagaaccaggacatgcccccccacctgccgacggccagcgcttccttccctgtacacccctactcctaccagtcgcctgggctgcccagtccgccttacggtaccatggacagctcccatgtcttccacgttaagcctccgccgcacgcctacagcgcagcgctggagcccttctttgaaagccctctgactgattgcaccagcccttcctttgatggacccctcagcccgccgctcagcatcaatggcaacttctctttcaaacacgaaccgtccgccgagtttgagaaaaattatgcctttaccatgcactatcctgcagcgacactggcaggggcccaaagccacggatcaatcttctcaggcaccgctgcccctcgctgcgagatccccatagacaatattatgtccttcgatagccattcacatcatgagcgagtcatgagtgcccagctcaatgccatatttcatgattag

SEQ ID NO: 2 - protein, 356 aa, Homo sapiens
  source 1..356: note = Human NeuroD1 Protein
MTKSYSESGLMGEPQPQGPPSWTDECLSSQDEEHEADKKEDDLETMNAEEDSLRNGGEEEDEDEDLEEEEEEEEEDDDQKPKRRGPKKKKMTKARLERFKLRRMKANARERNRMHGLNAALDNLRKVVPCYSKTQKLSKIETLRLAKNYIWALSEILRSGKSPDLVSFVQTLCKGLSQPTTNLVAGCLQLNPRTFLPEQNQDMPPHLPTASASFPVHPYSYQSPGLPSPPYGTMDSSHVFHVKPPPHAYSAALEPFFESPLTDCTSPSFDGPLSPPLSINGNFSFKHEPSAEFEKNYAFTMHYPAATLAGAQSHGSIFSGTAAPRCEIPIDNIMSFDSHSHHERVMSAQLNAIFHD

SEQ ID NO: 3 - DNA, 1071 bp, Homo sapiens
  source 1..1071: mol_type = other DNA; note = Human NeuroD1 Gene (CDS)
atgaccaaatcgtacagcgagagtgggctgatgggcgagcctcagccccaaggtcctccaagctggacagacgagtgtctcagttctcaggacgaggagcacgaggcagacaagaaggaggacgacctcgaaaccatgaacgcagaggaggactcactgaggaacgggggagaggaggaggacgaagatgaggacctggaagaggaggaagaagaggaagaggaggatgacgatcaaaagcccaagagacgcggccccaaaaagaagaagatgactaaggctcgcctggagcgttttaaattgagacgcatgaaggctaacgcccgggagcggaaccgcatgcacggactgaacgcggcgctagacaacctgcgcaaggtggtgccttgctattctaagacgcagaagctgtccaaaatcgagactctgcgcttggccaagaactacatctgggctctgtcggagatcctgcgctcaggcaaaagcccagacctggtctccttcgttcagacgctttgcaagggcttatcccaacccaccaccaacctggttgcgggctgcctgcaactcaatcctcggacttttctgcctgagcagaaccaggacatgcccccccacctgccgacggccagcgcttccttccctgtacacccctactcctaccagtcgcctgggctgcccagtccgccttacggtaccatggacagctcccatgtcttccacgttaagcctccgccgcacgcctacagcgcagcgctggagcccttctttgaaagccctctgactgattgcaccagcccttcctttgatggacccctcagcccgccgctcagcatcaatggcaacttctctttcaaacacgaaccgtccgccgagtttgagaaaaattatgcctttaccatgcactatcctgcagcgacactggcaggggcccaaagccacggatcaatcttctcaggcaccgctgcccctcgctgcgagatccccatagacaatattatgtccttcgatagccattcacatcatgagcgagtcatgagtgcccagctcaatgccatatttcatgattaa

SEQ ID NO: 4 - RNA, 1310 nt, Homo sapiens
  source 1..1310: mol_type = mRNA; note = Human NeuroD1 mRNA sequence
aggactcttctggtccccacagactcagagagaacccgccaccatgaccaaatcgtacagcgagagtgggctgatgggcgagcctcagccccaaggtcctccaagctggacagacgagtgtctcagttctcaggacgaggagcacgaggcagacaagaaggaggacgacctcgaaaccatgaacgcagaggaggactcactgaggaacgggggagaggaggaggacgaagatgaggacctggaagaggaggaagaagaggaagaggaggatgacgatcaaaagcccaagagacgcggccccaaaaagaagaagatgactaaggctcgcctggagcgttttaaattgagacgcatgaaggctaacgcccgggagcggaaccgcatgcacggactgaacgcggcgctagacaacctgcgcaaggtggtgccttgctattctaagacgcagaagctgtccaaaatcgagactctgcgcttggccaagaactacatctgggctctgtcggagatcctgcgctcaggcaaaagcccagacctggtctccttcgttcagacgctttgcaagggcttatcccaacccaccaccaacctggttgcgggctgcctgcaactcaatcctcggacttttctgcctgagcagaaccaggacatgcccccccacctgccgacggccagcgcttccttccctgtacacccctactcctaccagtcgcctgggctgcccagtccgccttacggtaccatggacagctcccatgtcttccacgttaagcctccgccgcacgcctacagcgcagcgctggagcccttctttgaaagccctctgactgattgcaccagcccttcctttgatggacccctcagcccgccgctcagcatcaatggcaacttctctttcaaacacgaaccgtccgccgagtttgagaaaaattatgcctttaccatgcactatcctgcagcgacactggcaggggcccaaagccacggatcaatcttctcaggcaccgctgcccctcgctgcgagatccccatagacaatattatgtccttcgatagccattcacatcatgagcgagtcatgagtgcccagctcaatgccatatttcatgattaatgataggctggagcctcggtggccatgcttcttgccccttgggcctccccccagcccctcctccccttcctgcacccgtacccccgtggtctttgaataaagtctgagtgggcggcaaaaaaaaaaaaaaaaaaaaaaaaaaaaaaaaaaaaaaaaaaaaaaaaaaaaaaaaaaaaaaaaaaaaaaaaaaaaaaaa

SEQ ID NO: 5 - RNA, 1310 nt, synthetic construct; identical to SEQ ID NO: 4
  source 1..1310: mol_type = other RNA; note = Human NeuroD1 mRNA containing modified nucleotides
  modified_base 6..1223: mod_base = m1f; note = all uridine bases are modified into N1-methyl pseudouridine(m1f)